European Patent Application EP 4 151 731 A1, published March 22, 2023. Title: Protein Composition Having Isoprene Polymerization Activity. Applicant: Sumitomo Riko Company Limited. The sequence listing filed with the application follows.

SEQUENCE LISTING (36 sequences)

SEQ ID NO: 1 - DNA, 873 bp, Hevea brasiliensis
atggaattatacaacggtgagaggccaagtgtgttcagacttttagggaagtatatgagaaaagggttatatagcatcctaacccagggtcccatccctactcatattgccttcatattggatggaaacaggaggtttgctaagaagcataaactgccagaaggaggtggtcataaggctggatttttagctcttctgaacgtactaacttattgctatgagttaggagtgaaatatgcgactatctatgcctttagcatcgataattttcgaaggaaacctcatgaggttcagtacgtaatggatctaatgctggagaagattgaagggatgatcatggaagaaagtatcatcaatgcatatgatatttgcgtacgttttgtgggtaacctgaagcttttaagtgagccagtcaagaccgcagcagataagattatgagggctactgccaacaattccaaatgtgtgcttctcattgctgtatgctatacttcaactgatgagatcgtgcatgctgttgaagaatcctctgaattgaactccaatgaagtttgtaacaatcaagaattggaggaggcaaatgcaactggaagcggtactgtgattcaaattgagaacatggagtcgtattctggaataaaacttgtagaccttgagaaaaacacctacataaatccttatcctgatgttctgattcgaacttctggggagacccgtctgagcaactacttactttggcagactactaattgcatactgtattctcctcatgcactgtggccagagattggtcttcgacacgtggtgtgggcagtaattaactgccaacgtcattattcttacttggagaaacataaggaatacttaaaataa

SEQ ID NO: 2 - protein, 290 aa, Hevea brasiliensis
MELYNGERPSVFRLLGKYMRKGLYSILTQGPIPTHIAFILDGNRRFAKKHKLPEGGGHKAGFLALLNVLTYCYELGVKYATIYAFSIDNFRRKPHEVQYVMDLMLEKIEGMIMEESIINAYDICVRFVGNLKLLSEPVKTAADKIMRATANNSKCVLLIAVCYTSTDEIVHAVEESSELNSNEVCNNQELEEANATGSGTVIQIENMESYSGIKLVDLEKNTYINPYPDVLIRTSGETRLSNYLLWQTTNCILYSPHALWPEIGLRHVVWAVINCQRHYSYLEKHKEYLK

SEQ ID NO: 3 - DNA, 891 bp, Hevea brasiliensis
atggaaatatatacgggtcagaggccaagtgtgtttagaatttttgggaaatacatgagaaaagggttatatagcatcctaacccaaggtcccatccctactcatcttgccttcataatggatggaaaccggaggtttgctaagaagcacaaaatgaaagaagcagaaggttataaggcaggatatttagctcttctgagaacactaacttattgctatgagttgggagtgaggtatgtaaccatttatgcctttagcattgataattttcgaaggcaacctcgtgaggttcagtgcgtaatgaatctaatgatggagaagattgaagagattatcgtggaagaaagtatcatgaatgcatatgatgttggcgtacgtattgtgggtaacctgaatcttttagatgagccaatcaggatcgcagcagaaaagattatgagggctactgccaataattccaggtttgtgcttctcattgctgtagcctatagttcaactgatgagatcgtgcatgctgttgaagaatcctctaaagacaaattgaactccaatgaagtttgcaacaatgggattgaagctgaacaagaatttaaggaggcaaacggaactggaaacagtgtgattccagttcagaagacggagtcatattctggaataaatcttgcagaccttgagaaaaacacctacgtaaatcctcatcctgatgtcttgattcgaacttctgggttgagccgtctaagtaactacctactttggcagactagtaattgcatactgtattctccttttgcactgtggccagagattggtctcaggcacttggtatggacagtaatgaacttccaacgtcatcattcttatttggagaagcataaggaatatttaaaataa

SEQ ID NO: 4 - protein, 296 aa, Hevea brasiliensis
MEIYTGQRPSVFRIFGKYMRKGLYSILTQGPIPTHLAFIMDGNRRFAKKHKMKEAEGYKAGYLALLRTLTYCYELGVRYVTIYAFSIDNFRRQPREVQCVMNLMMEKIEEIIVEESIMNAYDVGVRIVGNLNLLDEPIRIAAEKIMRATANNSRFVLLIAVAYSSTDEIVHAVEESSKDKLNSNEVCNNGIEAEQEFKEANGTGNSVIPVQKTESYSGINLADLEKNTYVNPHPDVLIRTSGLSRLSNYLLWQTSNCILYSPFALWPEIGLRHLVWTVMNFQRHHSYLEKHKEYLK

SEQ ID NO: 5 - DNA, 1122 bp, Hevea brasiliensis
atggaaaaacatagcagtagtagagtgagtgagctgtttggaaatttgggtagttttattagaatttgcatatttcgtgtgttatccatgggacccatccccaatcattttgccttcataatggatggaaatcggaggtatgctaagaaggagaacatgaaaaaaggggcaggtcatagggctggattcttagctcttatatccatacttaagtactgctatgaattgggagtgaagtatgtaacaatttacgcctttagcattgataatttcaaaaggagtcctgatgaagttaaggacctgatggatctgatgctagaaaagattgaggatttgctgagggacgaaagcattgtgaaccaatatggaatcagagtatattttataggtaatttgaaacttttgagtgaaactgtgaggattgcagcagaaaaggttatgaaagctactgccaaaaacaccaattgtacccttttaatctgcgtagcctatacgtcacgtgatgagattgtacatgctgttcaagtttcatgtaaaaataaacaggaggaaattcaaccattgagcttttgtaaagctaataatgatgccattgaagaagtagaggataataagaaggttaatggagtcatcccatttgtttttttagaatcccagaaagatgaagcaggcaaatctcaagcaacaatggcaagtgtaacctgcagttgtctggctagaggagttgaagggggtggcaacaaaaatagcatggttgttcgtgctgtccgaggatcctatgaagataaatgggataactgtcaagcaatgatggaaaatagaactggcaatggtgtgactttatctgaagagagtgagaatatgcagggagagtgttctatcataaagctagtagacattgagaaacagatgtacatggctgtagctcctgaacctgacatccttattcgaagttctggagagtcccgcctgagtaacttcctactttggcagaccagtgagtgccagttatattctccagatgcattgtggccagaaattggtttatggcacttggtgtgggcagtattaaacttccaacgaaaccatgcttatttggaaaagaaaaagcatcagttataa

SEQ ID NO: 6 - protein, 373 aa, Hevea brasiliensis
MEKHSSSRVSELFGNLGSFIRICIFRVLSMGPIPNHFAFIMDGNRRYAKKENMKKGAGHRAGFLALISILKYCYELGVKYVTIYAFSIDNFKRSPDEVKDLMDLMLEKIEDLLRDESIVNQYGIRVYFIGNLKLLSETVRIAAEKVMKATAKNTNCTLLICVAYTSRDEIVHAVQVSCKNKQEEIQPLSFCKANNDAIEEVEDNKKVNGVIPFVFLESQKDEAGKSQATMASVTCSCLARGVEGGGNKNSMVVRAVRGSYEDKWDNCQAMMENRTGNGVTLSEESENMQGECSIIKLVDIEKQMYMAVAPEPDILIRSSGESRLSNFLLWQTSECQLYSPDALWPEIGLWHLVWAVLNFQRNHAYLEKKKHQL

SEQ ID NO: 7 - DNA, 939 bp, Hevea brasiliensis
atgcaatccttgcacttggccctccctctccctttttacaacactctaactcctcaaaaacacaaacacttcctttctcccgatgccagaactaatacacgcccaattcaccgccttctcggggccaaaacagacgtagctgtcaaacaggaggaaactattgctgtaagcaccggagactcgcccaagactgaacctttgccggaggggctccggggagagttgatgccacggcatgtcgccgtgatcatggacggcaatgggaggtgggcccagctgcgaggtcagatggcatcgatgggtcatcaggctggtgcacggtctttgctggagatcgtgcagctttcttgtcaatgggggattaaagttcttagcgtttttgcgttttcttgcgataattggactaggcccaaagtcgtgcaggtggagattgatttcttgatgagtttgttcgaaagcgtgttaaagtcagagatggataaatttgtgagggaaggtattcgaatctctgtgatcggggactcatcaaggcttccacagtctttgcaaagattaataaatgaagtggaggagaccaccagaaatttctcgaaactgcaccttctagtggcggttagctacagtggaaagtatgatgttgtaaaagcatgcaaaagtattgcttgtctggtaaaggatggtgttattgaaccagaagacattagcgaaagcctaattgagcaggagttggaaacaaattgctccgagtttccctcccctgatttattaatccgaactagtggtgaacttagaattagcaacttcttgctatggcagttggcctacactgaacttttctttgcggaagaactctggcctgattttggaaaaactggattcatagaggccttaacttcataccaacaaaggcaaagacgctatggtagacgacttacataa

SEQ ID NO: 8 - protein, 312 aa, Hevea brasiliensis
MQSLHLALPLPFYNTLTPQKHKHFLSPDARTNTRPIHRLLGAKTDVAVKQEETIAVSTGDSPKTEPLPEGLRGELMPRHVAVIMDGNGRWAQLRGQMASMGHQAGARSLLEIVQLSCQWGIKVLSVFAFSCDNWTRPKVVQVEIDFLMSLFESVLKSEMDKFVREGIRISVIGDSSRLPQSLQRLINEVEETTRNFSKLHLLVAVSYSGKYDVVKACKSIACLVKDGVIEPEDISESLIEQELETNCSEFPSPDLLIRTSGELRISNFLLWQLAYTELFFAEELWPDFGKTGFIEALTSYQQRQRRYGRRLT

SEQ ID NO: 9 - DNA, 774 bp, Hevea brasiliensis
atggatttgaaacctggagctggagggcagagagttaatcgtttagtggatccgattagttatcattttcttcaatttctgtggcgtactctacatcttcttgtcagcttatggtaccttcaagttagtatggtccaaatgatcgaaggctttctaatctctagtggacttgtgaaacgctatggagccctcgatattgacaaggtccggtaccttgccattgtggtagatagtgaagaagcttaccaaatttctaaagttattcagcttttgaaatgggtggaagatatgggtgtgaaacatttatgcctctatgattcaaaaggagttctcaagacaaacaagaaaaccatcatggagagtttgaacaatgctatgccatttgaggaagcagttgaaaaagatgttttactggaccagaaacagatgactgtggaatttgcttccagctccgatggaaaggaagcaataaccagggcagctaacgtactctttatgaagtatttgaagtatgctaaaactggtgtaggaaaggaagaaccatgctttacagaagatcaaatggatgaggcactaaaagctataggttacaaagggccggaacctgacttgctattaatttatggacctgttagatgccatctaggtttctcaccgtggagacttcgatatactgagatggtgcatatgggacccttgaggtacatgaacctcggttcactaaaaaaggccattcacaggttcacaacagtgcagcaaaattatggtacataa

SEQ ID NO: 10 - protein, 257 aa, Hevea brasiliensis
MDLKPGAGGQRVNRLVDPISYHFLQFLWRTLHLLVSLWYLQVSMVQMIEGFLISSGLVKRYGALDIDKVRYLAIVVDSEEAYQISKVIQLLKWVEDMGVKHLCLYDSKGVLKTNKKTIMESLNNAMPFEEAVEKDVLLDQKQMTVEFASSSDGKEAITRAANVLFMKYLKYAKTGVGKEEPCFTEDQMDEALKAIGYKGPEPDLLLIYGPVRCHLGFSPWRLRYTEMVHMGPLRYMNLGSLKKAIHRFTTVQQNYGT

SEQ ID NO: 11 - DNA, 528 bp, Hevea brasiliensis
atggctgaaggtgaagaagaggtgaatatccaagaagaggcaaataaaggagaggagaatccccaagaagaggcgaatatccaagaagagacgaataaaggagaggagaatatccaagaagaggcgaatatcgaagaagaggctaataaggaggaagagagcctaaagtatttggattttgtgcaagcggctacagtttatgccagggcttctttctcaaagctctacctttttgccaaggacaagtctggtccattcaagcctggcgtcaatactgttgagagtaggtttaagagcgtggttagacccgtctataataagttccaacctgttcccaacaaggttctcaagtttgcagaccgtagggttgatgcatatgtcactgttttagatcgcattgttcctccaattgtcaagcgggcatctatccaagcttattcagtagccccaggagctgctcgtgctgtggcttcttatttgcctttgcataccaagagactttttaaggtgctatatggagatgggtga

SEQ ID NO: 12 - protein, 175 aa, Hevea brasiliensis
MAEGEEEVNIQEEANKGEENPQEEANIQEETNKGEENIQEEANIEEEANKEEESLKYLDFVQAATVYARASFSKLYLFAKDKSGPFKPGVNTVESRFKSVVRPVYNKFQPVPNKVLKFADRRVDAYVTVLDRIVPPIVKRASIQAYSVAPGAARAVASYLPLHTKRLFKVLYGDG

SEQ ID NO: 13 - DNA, 417 bp, Hevea brasiliensis
atggctgaagacgaagacaaccaacaagggcagggggaggggttaaaatatttgggttttgtgcaagacgcggcaacttatgctgtgactaccttctcaaacgtctatctttttgccaaagacaaatctggtccactgcagcctggtgtcgatatcattgagggtccggtgaagaacgtggctgtacctctctataataggttcagttatattcccaatggagctctcaagtttgtagacagcacggttgttgcatctgtcactattatagatcgctctcttcccccaattgtcaaggacgcatctatccaagttgtttcagcaattcgagctgccccagaagctgctcgttctctggcttcttctttgcctgggcagaccaagatacttgctaaggtgttttatggagagaattga

SEQ ID NO: 14 - protein, 138 aa, Hevea brasiliensis
MAEDEDNQQGQGEGLKYLGFVQDAATYAVTTFSNVYLFAKDKSGPLQPGVDIIEGPVKNVAVPLYNRFSYIPNGALKFVDSTVVASVTIIDRSLPPIVKDASIQVVSAIRAAPEAARSLASSLPGQTKILAKVFYGEN

SEQ ID NO: 15 - DNA, 354 bp, Hevea brasiliensis
atggctgaagggaaagaaaacgagaatttccaacaagaggctaatgagcaggaagagaagctaaagtatttggaatttgtacaagcgactacagataatgctgtaactgccctctcaaacatttacctttatgccaaggacaattctggtccgttgaagcctggggtcgagactattgagggtgtggcaaagaccgtggttattccggccagtaaaattcccactgaagctatcaagtttgcagacagagcggtggatgcatctttcactactctacaaaacattgttccctcagttctcaagcagttgcctacccaagcttgcgatactagtgtgaaggaaagtgcagagtaa

SEQ ID NO: 16 - protein, 117 aa, Hevea brasiliensis
MAEGKENENFQQEANEQEEKLKYLEFVQATTDNAVTALSNIYLYAKDNSGPLKPGVETIEGVAKTVVIPASKIPTEAIKFADRAVDASFTTLQNIVPSVLKQLPTQACDTSVKESAE

SEQ ID NO: 17 - DNA, 615 bp, Hevea brasiliensis
atggctgaagaggtggaggaagagaggctaaagtatttggattttgtgcgagcggctggagtttatgctgtagattctttctcaactctctacctttatgccaaggacatatctggtccattaaaacctggtgtcgatactattgagaatgtggtgaagaccgtggttactcctgtttattatattccccttgaggctgtcaagtttgtagacaaaacggtggatgtatcggtcactagcctagatggcgttgttcccccagttatcaagcaggtgtctgcccaaacttactcggtagctcaagatgctccaagaattgttcttgatgtggcttcttcagttttcaacactggtgtgcaggaaggcgcaaaagctctgtacgctaatcttgaaccaaaagctgagcaatatgcggtcattacctggcgtgccctcaataagctgccactagttcctcaagtggcaaatgtagttgtgccaaccgctgtttatttctctgaaaagtacaacgatgttgttcgtggcactactgagcagggatatagagtgtcctcttatttgcctttgttgcccactgagaaaattactaaggtgtttggagatgaggcatcataa

SEQ ID NO: 18 - protein, 204 aa, Hevea brasiliensis
MAEEVEEERLKYLDFVRAAGVYAVDSFSTLYLYAKDISGPLKPGVDTIENVVKTVVTPVYYIPLEAVKFVDKTVDVSVTSLDGVVPPVIKQVSAQTYSVAQDAPRIVLDVASSVFNTGVQEGAKALYANLEPKAEQYAVITWRALNKLPLVPQVANVVVPTAVYFSEKYNDVVRGTTEQGYRVSSYLPLLPTEKITKVFGDEAS

SEQ ID NO: 19 - DNA, 19 bp, Artificial Sequence
  Primer 1 for amplifying CPT1
atggaattatacaacggtg

SEQ ID NO: 20 - DNA, 36 bp, Artificial Sequence
  Primer 2 for amplifying CPT1
atctcgagttaatgatgatgatgatgatgttttaag

SEQ ID NO: 21 - DNA, 21 bp, Artificial Sequence
  Primer 3 for amplifying CPT2
atggaaatatatacgggtcag

SEQ ID NO: 22 - DNA, 41 bp, Artificial Sequence
  Primer 4 for amplifying CPT2
atctcgagttaatgatgatgatgatgatgttttaaatattc

SEQ ID NO: 23 - DNA, 20 bp, Artificial Sequence
  Primer 5 for amplifying CPT6
atggaaaaacatagcagtag

SEQ ID NO: 24 - DNA, 29 bp, Artificial Sequence
  Primer 6 for amplifying CPT6
atctcgagttatataactgatgctttttc

SEQ ID NO: 25 - DNA, 18 bp, Artificial Sequence
  Primer 7 for amplifying CPT7
atgcaatccttgcacttg

SEQ ID NO: 26 - DNA, 30 bp, Artificial Sequence
  Primer 8 for amplifying CPT7
atctcgagttatgtaagtcgtctaccatag

SEQ ID NO: 27 - DNA, 17 bp, Artificial Sequence
  Primer 9 for amplifying CPTL
atggatttgaaacctgg

SEQ ID NO: 28 - DNA, 34 bp, Artificial Sequence
  Primer 10 for amplifying CPTL
atctcgagttaatgatgatgatgatgatgtgtac

SEQ ID NO: 29 - DNA, 30 bp, Artificial Sequence
  Primer 11 for amplifying REF1
atggctgaaggtgaagaagaggtgaatatc

SEQ ID NO: 30 - DNA, 29 bp, Artificial Sequence
  Primer 12 for amplifying REF1
atctcgagtcacccatctccatatagcac

SEQ ID NO: 31 - DNA, 28 bp, Artificial Sequence
  Primer 13 for amplifying REF2
atggctgaagacgaagacaaccaacaag

SEQ ID NO: 32 - DNA, 29 bp, Artificial Sequence
  Primer 14 for amplifying REF2
atctcgagtcaattctctccataaaacac

SEQ ID NO: 33 - DNA, 30 bp, Artificial Sequence
  Primer 15 for amplifying REF8
atggctgaagggaaagaaaacgagaatttc

SEQ ID NO: 34 - DNA, 29 bp, Artificial Sequence
  Primer 16 for amplifying REF8
atctcgagttactctgcactttccttcac

SEQ ID NO: 35 - DNA, 28 bp, Artificial Sequence
  Primer 17 for amplifying SRPP1
atggctgaagaggtggaggaagagaggc

SEQ ID NO: 36 - DNA, 30 bp, Artificial Sequence
  Primer 18 for amplifying SRPP1
atctcgagttatgatgcctcatctccaaac